European Patent Application EP 4 428 154 A1, published September 11, 2024. Title: ANTI-CLDN18.2 ANTIBODY AND USE THEREOF. Applicant: Chia Tai Tianqing Pharmaceutical Group Co., Ltd. The sequence listing filed with the application follows.

SEQUENCE LISTING (68 sequences)

SEQ ID NO: 1 - protein, 261 aa, Homo sapiens
  source 1..261: note = human CLDN18.2
MAVTACQGLGFVVSLIGIAGIIAATCMDQWSTQDLYNNPVTAVFNYQGLWRSCVRESSGFTECRGYFTLLGLPAMLQAVRALMIVGIVLGAIGLLVSIFALKCIRIGSMEDSAKANMTLTSGIMFIVSGLCAIAGVSVFANMLVTNFWMSTANMYTGMGGMVQTVQTRYTFGAALFVGWVAGGLTLIGGVMMCIACRGLAPEETNYKAVSYHASGHSVAYKPGGFKASTGFGSNTKNKKIYDGGARTEDEVQSYPSKHDYV

SEQ ID NO: 2 - protein, 261 aa, Homo sapiens
  source 1..261: note = human CLDN18.1
MSTTTCQVVAFLLSILGLAGCIAATGMDMWSTQDLYDNPVTSVFQYEGLWRSCVRQSSGFTECRPYFTILGLPAMLQAVRALMIVGIVLGAIGLLVSIFALKCIRIGSMEDSAKANMTLTSGIMFIVSGLCAIAGVSVFANMLVTNFWMSTANMYTGMGGMVQTVQTRYTFGAALFVGWVAGGLTLIGGVMMCIACRGLAPEETNYKAVSYHASGHSVAYKPGGFKASTGFGSNTKNKKIYDGGARTEDEVQSYPSKHDYV

SEQ ID NO: 3 - protein, 5 aa, synthetic construct
  source 1..5: note = HCDR1 of mouse, chimeric, and humanized 28G3
DYLML

SEQ ID NO: 4 - protein, 17 aa, synthetic construct
  source 1..17: note = HCDR2 of mouse and chimeric 28G3
NINPYYGRTTYNLKFKG

SEQ ID NO: 5 - protein, 17 aa, synthetic construct
  source 1..17: note = HCDR2 of hz28G3-1.1, hz28G3-1.3, hz28G3-2.1, and hz28G3-2.3
NINPYYGRTTYALKFKG

SEQ ID NO: 6 - protein, 17 aa, synthetic construct
  source 1..17: note = HCDR2 of hz28G3-1.2, hz28G3-1.4, hz28G3-2.2, and hz28G3-2.4
NINPYYGRTYYALKFQG

SEQ ID NO: 7 - protein, 11 aa, synthetic construct
  source 1..11: note = HCDR3 of mouse, chimeric, and humanized 28G3
DGYSLRNAMDY

SEQ ID NO: 8 - protein, 17 aa, synthetic construct
  source 1..17: note = LCDR1 of mouse, chimeric, and humanized 28G3
KSSQSLFNSGNQKNYLA

SEQ ID NO: 9 - protein, 7 aa, synthetic construct
  source 1..7: note = LCDR2 of mouse, chimeric, and humanized 28G3
GASTRES

SEQ ID NO: 10 - protein, 9 aa, synthetic construct
  source 1..9: note = LCDR3 of mouse, chimeric, and humanized 28G3
QNAHSYPYT

SEQ ID NO: 11 - protein, 120 aa, synthetic construct
  source 1..120: note = VH of mouse and chimeric 28G3
EIQLQQTGPELVKPGASVTISCKTSGYSFTDYLMLWVKQSHGKSLEWIGNINPYYGRTTYNLKFKGKATLTVDRSSSTAYMQLNSLTSEDSAVYYCARDGYSLRNAMDYWGQGTSVTVSS

SEQ ID NO: 12 - protein, 120 aa, synthetic construct
  source 1..120: note = VH of hz28G3-1.1 and hz28G3-2.1
QVQLVQSGAEVKKPGASVKVSCKTSGYSFTDYLMLWVRQAPGQGLEWMGNINPYYGRTTYALKFKGRVTMTVDRSTSTVYMELSSLRSEDTAVYYCARDGYSLRNAMDYWGQGTLVTVSS

SEQ ID NO: 13 - protein, 120 aa, synthetic construct
  source 1..120: note = VH of hz28G3-1.2 and hz28G3-2.2
QVQLVQSGAEVKKPGASVKVSCKASGYTFTDYLMLWVRQAPGQGLEWMGNINPYYGRTYYALKFQGRVTMTVDRSTSTVYMELSSLRSEDTAVYYCARDGYSLRNAMDYWGQGTLVTVSS

SEQ ID NO: 14 - protein, 120 aa, synthetic construct
  source 1..120: note = VH of hz28G3-1.3 and hz28G3-2.3
QVQLVQSGAEVKKPGASVKVSCKTSGYSFTDYLMLWVRQAHGQSLEWMGNINPYYGRTTYALKFKGRVTMTVDRSTSTVYMELSSLRSEDTAVYYCARDGYSLRNAMDYWGQGTLVTVSS

SEQ ID NO: 15 - protein, 120 aa, synthetic construct
  source 1..120: note = VH of hz28G3-1.4 and hz28G3-2.4
QVQLVQSGAEVKKPGASVKVSCKASGYTFTDYLMLWVRQAHGQSLEWMGNINPYYGRTYYALKFQGRVTMTVDRSTSTVYMELSSLRSEDTAVYYCARDGYSLRNAMDYWGQGTLVTVSS

SEQ ID NO: 16 - protein, 113 aa, synthetic construct
  source 1..113: note = VL of mouse and chimeric 28G3
DIVMTQSPYSLSVSTGEKVTMSCKSSQSLFNSGNQKNYLAWYQQKPGQPPKLLIYGASTRESGVPDRFTGSGSGTDFTLTISSVQAEDLALYYCQNAHSYPYTFGGGTKLEIK

SEQ ID NO: 17 - protein, 113 aa, synthetic construct
  source 1..113: note = VL of hz28G3-1.1, hz28G3-1.2, hz28G3-1.3, and hz28G3-1.4
DIVMTQSPDSLAVSLGERATINCKSSQSLFNSGNQKNYLAWYQQKPGQPPKLLIYGASTRESGVPDRFSGSGSGTDFTLTISSLQAEDVAVYYCQNAHSYPYTFGQGTKVEIK

SEQ ID NO: 18 - protein, 113 aa, synthetic construct
  source 1..113: note = VL of hz28G3-2.1, hz28G3-2.2, hz28G3-2.3, and hz28G3-2.4
DIVMTQSPYSLAVSLGERATINCKSSQSLFNSGNQKNYLAWYQQKPGQPPKLLIYGASTRESGVPDRFTGSGSGTDFTLTISSLQAEDVAVYYCQNAHSYPYTFGQGTKVEIK

SEQ ID NO: 19 - protein, 5 aa, synthetic construct
  source 1..5: note = HCDR1 of mouse, chimeric, and humanized 40F6
SYGVY

SEQ ID NO: 20 - protein, 16 aa, synthetic construct
  source 1..16: note = HCDR2 of mouse and chimeric 40F6, hz40F6-1.2, and hz40F6-2.2
VVWAGGNTNYNSALMS

SEQ ID NO: 21 - protein, 16 aa, synthetic construct
  source 1..16: note = HCDR2 of hz40F6-1.1 and hz40F6-2.1
VVWAGGNTNYADSVKG

SEQ ID NO: 22 - protein, 16 aa, synthetic construct
  source 1..16: note = HCDR2 of hz40F6-1.3 and hz40F6-2.3
VVWAGGNTNYADALKG

SEQ ID NO: 23 - protein, 16 aa, synthetic construct
  source 1..16: note = HCDR2 of hz40F6-1.4 and hz40F6-2.4
VVWAGGNTNYNSALKG

SEQ ID NO: 24 - protein, 10 aa, synthetic construct
  source 1..10: note = HCDR3 of mouse, chimeric, and humanized 40F6
DRGRLLAMDY

SEQ ID NO: 25 - protein, 17 aa, synthetic construct
  source 1..17: note = LCDR1 of mouse, chimeric, and humanized 40F6
KSSQSLLNSGNQKNYLA

SEQ ID NO: 26 - protein, 7 aa, synthetic construct
  source 1..7: note = LCDR2 of mouse, chimeric, and humanized 40F6
GASTRES

SEQ ID NO: 27 - protein, 9 aa, synthetic construct
  source 1..9: note = LCDR3 of mouse and chimeric 40F6, hz40F6-1.1, hz40F6-1.2, hz40F6-1.3, and hz40F6-1.4
QNDHFFPFT

SEQ ID NO: 28 - protein, 9 aa, synthetic construct
  source 1..9: note = LCDR3 of hz40F6-2.1, hz40F6-2.2, hz40F6-2.3, and hz40F6-2.4
QNDYFFPFT

SEQ ID NO: 29 - protein, 118 aa, synthetic construct
  source 1..118: note = VH of mouse and chimeric 40F6
QVQLKESGPGLVAPSQSLSITCTVSGFSLTSYGVYWVRQSPGKGLEWLGVVWAGGNTNYNSALMSRLSISKDNSKSQVFLKMNSLQTDDTAMYYCARDRGRLLAMDYWGQGTSVTVSS

SEQ ID NO: 30 - protein, 118 aa, synthetic construct
  source 1..118: note = VH of hz40F6-1.1 and hz40F6-2.1
QVQLVESGGGVVQPGRSLRLSCAASGFTLTSYGVYWVRQAPGKGLEWVAVVWAGGNTNYADSVKGRFTISKDNSKSTLYLQMNSLRAEDTAVYYCARDRGRLLAMDYWGQGTLVTVSS

SEQ ID NO: 31 - protein, 118 aa, synthetic construct
  source 1..118: note = VH of hz40F6-1.2 and hz40F6-2.2
QVQLVESGGGVVQPGRSLRLSCAASGFTLTSYGVYWVRQAPGKGLEWVAVVWAGGNTNYNSALMSRFTISKDNSKSTLYLQMNSLRAEDTAVYYCARDRGRLLAMDYWGQGTLVTVSS

SEQ ID NO: 32 - protein, 118 aa, synthetic construct
  source 1..118: note = VH of hz40F6-1.3 and hz40F6-2.3
QVQLVESGGGVVQPGRSLRLSCAASGFTLTSYGVYWVRQAPGKGLEWVAVVWAGGNTNYADALKGRFTISKDNSKSTLYLQMNSLRAEDTAVYYCARDRGRLLAMDYWGQGTLVTVSS

SEQ ID NO: 33 - protein, 118 aa, synthetic construct
  source 1..118: note = VH of hz40F6-1.4 and hz40F6-2.4
QVQLVESGGGVVQPGRSLRLSCTVSGFTLTSYGVYWVRQAPGKGLEWVAVVWAGGNTNYNSALKGRFTISKDNSKSTLYLQMNSLRAEDTAVYYCARDRGRLLAMDYWGQGTLVTVSS

SEQ ID NO: 34 - protein, 113 aa, synthetic construct
  source 1..113: note = VL of mouse and chimeric 40F6
DVVMTQSPSSLSVSAGEKVTMSCKSSQSLLNSGNQKNYLAWYQQKPGQPPKLLIYGASTRESGVPDRFTGSGSGTDFTLTISSVQAEDLAVYYCQNDHFFPFTFGSGTKLEIK

SEQ ID NO: 35 - protein, 113 aa, synthetic construct
  source 1..113: note = VL of hz40F6-1.1, hz40F6-1.2, hz40F6-1.3, and hz40F6-1.4
DIVMTQSPDSLAVSLGERATINCKSSQSLLNSGNQKNYLAWYQQKPGQPPKLLIYGASTRESGVPDRFTGSGSGTDFTLTISSLQAEDVAVYYCQNDHFFPFTFGQGTKVEIK

SEQ ID NO: 36 - protein, 113 aa, synthetic construct
  source 1..113: note = VL of hz40F6-2.1, hz40F6-2.2, hz40F6-2.3, and hz40F6-2.4
DIVMTQSPDSLAVSLGERATINCKSSQSLLNSGNQKNYLAWYQQKPGQPPKLLIYGASTRESGVPDRFSGSGSGTDFTLTISSLQAEDVAVYYCQNDYFFPFTFGQGTKVEIK

SEQ ID NO: 37 - protein, 5 aa, synthetic construct
  source 1..5: note = HCDR1 of mouse and chimeric 34G6
SYGVH

SEQ ID NO: 38 - protein, 16 aa, synthetic construct
  source 1..16: note = HCDR2 of mouse and chimeric 34G6
VIWSDGSTTYNSALKS

SEQ ID NO: 39 - protein, 10 aa, synthetic construct
  source 1..10: note = HCDR3 of mouse and chimeric 34G6
HAYYGNSFDY

SEQ ID NO: 40 - protein, 17 aa, synthetic construct
  source 1..17: note = LCDR1 of mouse and chimeric 34G6
KSSQSLLNSGNQKSYLT

SEQ ID NO: 41 - protein, 7 aa, synthetic construct
  source 1..7: note = LCDR2 of mouse and chimeric 34G6
WASTRES

SEQ ID NO: 42 - protein, 9 aa, synthetic construct
  source 1..9: note = LCDR3 of mouse and chimeric 34G6
QNVYIFPLT

SEQ ID NO: 43 - protein, 118 aa, synthetic construct
  source 1..118: note = VH of mouse and chimeric 34G6
QVQLKESGPDLVAPSQSLSITCTVSGFSLTSYGVHWVRQPPGKGLEWLVVIWSDGSTTYNSALKSRLSISKDNSKSQVFLKMNSLQTDDTAIYYCARHAYYGNSFDYWGQGTTLTVSS

SEQ ID NO: 44 - protein, 113 aa, synthetic construct
  source 1..113: note = VL of mouse and chimeric 34G6
DIVMTQSPSSLTVTAGEKVTMSCKSSQSLLNSGNQKSYLTWYQQKPGQPPKLLIYWASTRESGVPDRFTGSGSGTDFTLTISSVQAEDLAVYYCQNVYIFPLTFGAGTKLELK

SEQ ID NO: 45 - protein, 5 aa, synthetic construct
  source 1..5: note = HCDR1 of mouse and chimeric 10D8
NYGMN

SEQ ID NO: 46 - protein, 17 aa, synthetic construct
  source 1..17: note = HCDR2 of mouse and chimeric 10D8
WININTGEPRYAEEFKG

SEQ ID NO: 47 - protein, 9 aa, synthetic construct
  source 1..9: note = HCDR3 of mouse and chimeric 10D8
YGYGNSFPY

SEQ ID NO: 48 - protein, 17 aa, synthetic construct
  source 1..17: note = LCDR1 of mouse and chimeric 10D8
KSSQSLLNSGNQRNYLT

SEQ ID NO: 49 - protein, 7 aa, synthetic construct
  source 1..7: note = LCDR2 of mouse and chimeric 10D8
WASTRES

SEQ ID NO: 50 - protein, 9 aa, synthetic construct
  source 1..9: note = LCDR3 of mouse and chimeric 10D8
QNDYSYPLT

SEQ ID NO: 51 - protein, 118 aa, synthetic construct
  source 1..118: note = VH of mouse and chimeric 10D8
QIQLAQSGPELKKPGETVKVSCKASGYTFKNYGMNWVKQAPGKGLKWMGWININTGEPRYAEEFKGRIAFSLETSASTAYLLINNLKNEDTATYFCARYGYGNSFPYWGQGTLVTVSA

SEQ ID NO: 52 - protein, 113 aa, synthetic construct
  source 1..113: note = VL of mouse and chimeric 10D8
DIVMTQSPSSLTVTVGEKVTMSCKSSQSLLNSGNQRNYLTWYQQKPGQPPKLLIYWASTRESGVPDRFTGSGSGTAFTLTVSSVQAEDLAVYYCQNDYSYPLTFGAGTKLEMK

SEQ ID NO: 53 - protein, 5 aa, synthetic construct
  source 1..5: note = HCDR1 of mouse and chimeric 22F12
SYGVY

SEQ ID NO: 54 - protein, 16 aa, synthetic construct
  source 1..16: note = HCDR2 of mouse and chimeric 22F12
VIWAGGSTNYNSALMS

SEQ ID NO: 55 - protein, 10 aa, synthetic construct
  source 1..10: note = HCDR3 of mouse and chimeric 22F12
DRGRLLSMDY

SEQ ID NO: 56 - protein, 17 aa, synthetic construct
  source 1..17: note = LCDR1 of mouse and chimeric 22F12
RSSQSLLNSGNQKNYLA

SEQ ID NO: 57 - protein, 7 aa, synthetic construct
  source 1..7: note = LCDR2 of mouse and chimeric 22F12
GASTRES

SEQ ID NO: 58 - protein, 9 aa, synthetic construct
  source 1..9: note = LCDR3 of mouse and chimeric 22F12
QNVHFFPFT

SEQ ID NO: 59 - protein, 118 aa, synthetic construct
  source 1..118: note = VH of mouse and chimeric 22F12
QVQLKESGPGLVAPSQSLSITCTVSGFSLTSYGVYWVRQPPGKGLEWLGVIWAGGSTNYNSALMSRLSINKDNSKSQVFLKMNSLQTDDTAMYYCARDRGRLLSMDYWGQGTSVTVSS

SEQ ID NO: 60 - protein, 113 aa, synthetic construct
  source 1..113: note = VL of mouse and chimeric 22F12
DIVMTQSPSSLSVSAGEKVTMSCRSSQSLLNSGNQKNYLAWYQQKPGQPPKLLIYGASTRESGVPDRFTGSGSGTDFTLTIGSVQAEDLAVYYCQNVHFFPFTFGSGTKLEIK

SEQ ID NO: 61 - protein, 330 aa, synthetic construct [sequence omitted]

SEQ ID NO: 62 - protein, 107 aa, synthetic construct [sequence omitted]

SEQ ID NO: 63 - protein, 448 aa, synthetic construct
  source 1..448: note = Heavy chain of IMAB362
QVQLQQPGAELVRPGASVKLSCKASGYTFTSYWINWVKQRPGQGLEWIGNIYPSDSYTNYNQKFKDKATLTVDKSSSTAYMQLSSPTSEDSAVYYCTRSWRGNSFDYWGQGTTLTVSSASTKGPSVFPLAPSSKSTSGGTAALGCLVKDYFPEPVTVSWNSGALTSGVHTFPAVLQSSGLYSLSSVVTVPSSSLGTQTYICNVNHKPSNTKVDKKVEPKSCDKTHTCPPCPAPELLGGPSVFLFPPKPKDTLMISRTPEVTCVVVDVSHEDPEVKFNWYVDGVEVHNAKTKPREEQYNSTYRVVSVLTVLHQDWLNGKEYKCKVSNKALPAPIEKTISKAKGQPREPQVYTLPPSRDELTKNQVSLTCLVKGFYPSDIAVEWESNGQPENNYKTTPPVLDSDGSFFLYSKLTVDKSRWQQGNVFSCSVMHEALHNHYTQKSLSLSPGK

SEQ ID NO: 64 - protein, 220 aa, synthetic construct
  source 1..220: note = Light chain of IMAB362
DIVMTQSPSSLTVTAGEKVTMSCKSSQSLLNSGNQKNYLTWYQQKPGQPPKLLIYWASTRESGVPDRFTGSGSGTDFTLTISSVQAEDLAVYYCQNDYSYPFTFGSGTKLEIKRTVAAPSVFIFPPSDEQLKSGTASVVCLLNNFYPREAKVQWKVDNALQSGNSQESVTEQDSKDSTYSLSSTLTLSKADYEKHKVYACEVTHQGLSSPVTKSFNRGEC

SEQ ID NO: 65 - protein, 448 aa, synthetic construct
  source 1..448: note = Heavy chain of 15F9
QVQLVQSGSELKKPGASVKVSCKASGYTFTNYGINWVRQAPGQGLEWMGWINPNTGETTYAEEFKGRFVFSLDTSVSTAYLQISSLKAEDTAVYFCARLYYGNRFDSWGQGTLVTVSSASTKGPSVFPLAPSSKSTSGGTAALGCLVKDYFPEPVTVSWNSGALTSGVHTFPAVLQSSGLYSLSSVVTVPSSSLGTQTYICNVNHKPSNTKVDKKVEPKSCDKTHTCPPCPAPELLGGPSVFLFPPKPKDTLMISRTPEVTCVVVDVSHEDPEVKFNWYVDGVEVHNAKTKPREEQYNSTYRVVSVLTVLHQDWLNGKEYKCKVSNKALPAPIEKTISKAKGQPREPQVYTLPPSRDELTKNQVSLTCLVKGFYPSDIAVEWESNGQPENNYKTTPPVLDSDGSFFLYSKLTVDKSRWQQGNVFSCSVMHEALHNHYTQKSLSLSPGK

SEQ ID NO: 66 - protein, 220 aa, synthetic construct
  source 1..220: note = Light chain of 15F9
DIVMTQSPDSLAVSLGERATINCKSSQSLLNSGNQRNYLTWYQQKPGQPPKLLIYWASTRESGVPDRFSGSGSGTDFTLTISSLQAEDVAVYYCQNAYYYPLTFGGGTKVEIKRTVAAPSVFIFPPSDEQLKSGTASVVCLLNNFYPREAKVQWKVDNALQSGNSQESVTEQDSKDSTYSLSSTLTLSKADYEKHKVYACEVTHQGLSSPVTKSFNRGEC

SEQ ID NO: 67 - protein, 446 aa, synthetic construct
  source 1..446: note = Heavy chain of IgG1 isotype control antibody
EVQLEQSGAELMKPGASVKISCKATGYTFTTYWIEWIKQRPGHSLEWIGEILPGSDSTYYNEKVKGKVTFTADASSNTAYMQLSSLTSEDSAVYYCARGDGFYVYWGQGTTLTVSSASTKGPSVFPLAPSSKSTSGGTAALGCLVKDYFPEPVTVSWNSGALTSGVHTFPAVLQSSGLYSLSSVVTVPSSSLGTQTYICNVNHKPSNTKVDKKVEPKSCDKTHTCPPCPAPELLGGPSVFLFPPKPKDTLMISRTPEVTCVVVDVSHEDPEVKFNWYVDGVEVHNAKTKPREEQYNSTYRVVSVLTVLHQDWLNGKEYKCKVSNKALPAPIEKTISKAKGQPREPQVYTLPPSRDELTKNQVSLTCLVKGFYPSDIAVEWESNGQPENNYKTTPPVLDSDGSFFLYSKLTVDKSRWQQGNVFSCSVMHEALHNHYTQKSLSLSPGK

SEQ ID NO: 68 - protein, 214 aa, synthetic construct
  source 1..214: note = Light chain of IgG1 isotype control antibody
DIELTQSPATLSVTPGDSVSLSCRASQSISNNLHWYQQKSHESPRLLIKYTSQSMSGIPSRFSGSGSGTDFTLSINSVETEDFGVYFCQQSGSWPRTFGGGTKLDIKRTVAAPSVFIFPPSDEQLKSGTASVVCLLNNFYPREAKVQWKVDNALQSGNSQESVTEQDSKDSTYSLSSTLTLSKADYEKHKVYACEVTHQGLSSPVTKSFNRGEC